European Patent Application EP 4 628 579 A1, published October 8, 2025. Title: TRANSAMINASE MUTANT AND USE. Applicant: ASYMCHEM LIFE SCIENCE(TIANJIN)CO,.LTD. Application CN. The sequence listing filed with the application follows.

SEQUENCE LISTING (1 sequence)

SEQ ID NO: 1 - protein, 459 aa, Chromobacterium violaceum
MQKQRTCSQWRELDAAHHLHPFTDTASLNQVGARVMTRGEGVYLWDCEGNKIIDGMAGAWCVNMGYGRKDFAEAARRQMEELSFMHTADGITHPAVVELSSLLAEVTPAGFDRVFYTNSGSESVDCMIRMVRRYWDVQGKPEKKTLIGRWNGYSGSTIGGASLSGFKEMHEQGDLPIPGVAHIEQPWWYKHGKDMTPDEFGVVAARWLEEKILEIGADKVAAFVGEPIQGAGGAIVPPATYWPEIERICRKYDVLLVADEVICGFGRTGEWFGHQHFGFQPDLFTAAKGLSSGYQPIGAVSVGKRVAEGLIAGGVFYHGHTTSGHPVCAAVAHANVAALRDEGIVQRVKDDIGPYMQKRWRETLSRFEHVDDVRGVGMLAAFTLVKNKAKRELFPDFGEIGSLCRDIFVRNNLIMDICGDHIVAAPPLVMTRAEVDEMLAVAERCLEELEQSLKARGLA